European Patent Application EP 4 806 917 A1, published September 16, 2026. Title: 靶向B7H3抗原结合蛋白及其应用. Applicant: 重庆茂行生命健康科技有限公司. Application WO. The sequence listing filed with the application follows.

SEQUENCE LISTING (29 sequences)

SEQ ID NO: 1 - protein, 5 aa, synthetic construct
  REGION 1..5: note = HCDR1
NYAMG

SEQ ID NO: 2 - protein, 16 aa, synthetic construct
  REGION 1..16: note = HCDR2
VIGGSGNTYYARWAKG

SEQ ID NO: 3 - protein, 16 aa, synthetic construct
  REGION 1..16: note = HCDR3
GGADIHGYAYGTLGTL

SEQ ID NO: 4 - protein, 11 aa, synthetic construct
  REGION 1..11: note = LCDR1
QASQSIGTALA

SEQ ID NO: 5 - protein, 7 aa, synthetic construct
  REGION 1..7: note = LCDR2
YASTLAS

SEQ ID NO: 6 - protein, 14 aa, synthetic construct
  REGION 1..14: note = LCDR3
QSYYYSNNNSDGSA

SEQ ID NO: 7 - protein, 8 aa, synthetic construct
  REGION 1..8: note = HCDR1
GIDLSNYA

SEQ ID NO: 8 - protein, 7 aa, synthetic construct
  REGION 1..7: note = HCDR2
IGGSGNT

SEQ ID NO: 9 - protein, 18 aa, synthetic construct
  REGION 1..18: note = HCDR3
ARGGADIHGYAYGTLGTL

SEQ ID NO: 10 - protein, 6 aa, synthetic construct
  REGION 1..6: note = LCDR1
QSIGTA

SEQ ID NO: 11 - skipped

SEQ ID NO: 12 - protein, 7 aa, synthetic construct
  REGION 1..7: note = HCDR1
GIDLSNY

SEQ ID NO: 13 - protein, 5 aa, synthetic construct
  REGION 1..5: note = HCDR2
GGSGN

SEQ ID NO: 14 - protein, 6 aa, synthetic construct
  REGION 1..6: note = HCDR1
SNYAMG

SEQ ID NO: 15 - protein, 12 aa, synthetic construct
  REGION 1..12: note = HCDR2
YIGVIGGSGNTY

SEQ ID NO: 16 - protein, 17 aa, synthetic construct
  REGION 1..17: note = HCDR3
ARGGADIHGYAYGTLGT

SEQ ID NO: 17 - protein, 7 aa, synthetic construct
  REGION 1..7: note = LCDR1
GTALAWY

SEQ ID NO: 18 - protein, 10 aa, synthetic construct
  REGION 1..10: note = LCDR2
LLIYYASTLA

SEQ ID NO: 19 - protein, 13 aa, synthetic construct
  REGION 1..13: note = LCDR3
QSYYYSNNNSDGS

SEQ ID NO: 20 - protein, 121 aa, synthetic construct
  REGION 1..121: note = VH
QSLEESGGRLVTPGTPLTLTCAGSGIDLSNYAMGWVRQAPGKGLEYIGVIGGSGNTYYARWAKGRFTISKTSTTVDLKITSPTTEDTATYFCARGGADIHGYAYGTLGTLWGPGTLVTVSS

SEQ ID NO: 21 - protein, 113 aa, synthetic construct
  REGION 1..113: note = VL
ADIVMTQTPASVEAAVGGTVTIKCQASQSIGTALAWYQQKPGQPPKLLIYYASTLASGVPSRFKGSGSGTQFTFTISDLECADAATYYCQSYYYSNNNSDGSAFGGGTEVVVK

SEQ ID NO: 22 - protein, 323 aa, synthetic construct
GQPKAPSVFPLAPCCGDTPSSTVTLGCLVKGYLPEPVTVTWNSGTLTNGVRTFPSVRQSSGLYSLSSVVSVTSSSQPVTCNVAHPATNTKVDKTVAPSTCSKPTCPPPELLGGPSVFIFPPKPKDTLMISRTPEVTCVVVDVSQDDPEVQFTWYINNEQVRTARPPLREQQFNSTIRVVSTLPIAHQDWLRGKEFKCKVHNKALPAPIEKTISKARGQPLEPKVYTMGPPREELSSRSVSLTCMINGFYPSDISVEWEKNGKAEDNYKTTPAVLDSDGSYFLYSKLSVPTSEWQRGDVFTCSVMHEALHNHYTQKSISRSPGK

SEQ ID NO: 23 - protein, 104 aa, synthetic construct
GDPVAPTVLIFPPAADQVATGTVTIVCVANKYFPDVTVTWEVDGTTQTTGIENSKTPQNSADCTYNLSSTLTLTSTQYNSHKEYTCKVTQGTTSVVQSFNRGDC

SEQ ID NO: 24 - protein, 444 aa, synthetic construct
  REGION 1..444: note = HC
QSLEESGGRLVTPGTPLTLTCAGSGIDLSNYAMGWVRQAPGKGLEYIGVIGGSGNTYYARWAKGRFTISKTSTTVDLKITSPTTEDTATYFCARGGADIHGYAYGTLGTLWGPGTLVTVSSGQPKAPSVFPLAPCCGDTPSSTVTLGCLVKGYLPEPVTVTWNSGTLTNGVRTFPSVRQSSGLYSLSSVVSVTSSSQPVTCNVAHPATNTKVDKTVAPSTCSKPTCPPPELLGGPSVFIFPPKPKDTLMISRTPEVTCVVVDVSQDDPEVQFTWYINNEQVRTARPPLREQQFNSTIRVVSTLPIAHQDWLRGKEFKCKVHNKALPAPIEKTISKARGQPLEPKVYTMGPPREELSSRSVSLTCMINGFYPSDISVEWEKNGKAEDNYKTTPAVLDSDGSYFLYSKLSVPTSEWQRGDVFTCSVMHEALHNHYTQKSISRSPGK

SEQ ID NO: 25 - protein, 217 aa, synthetic construct
  REGION 1..217: note = LC
ADIVMTQTPASVEAAVGGTVTIKCQASQSIGTALAWYQQKPGQPPKLLIYYASTLASGVPSRFKGSGSGTQFTFTISDLECADAATYYCQSYYYSNNNSDGSAFGGGTEVVVKGDPVAPTVLIFPPAADQVATGTVTIVCVANKYFPDVTVTWEVDGTTQTTGIENSKTPQNSADCTYNLSSTLTLTSTQYNSHKEYTCKVTQGTTSVVQSFNRGDC

SEQ ID NO: 26 - DNA, 1332 bp, synthetic construct
  misc_feature 1..1332: note = HC DNA
  source 1..1332: mol_type = other DNA
cagtcgctggaggagtccgggggtcgcctggtcacgcctgggacacccctgacactcacctgcgctggctctggaatcgacctcagtaactatgcaatgggctgggtccgccaggctccagggaaggggctggaatacatcggagtcattggtggtagtggtaacacatactacgcgaggtgggcgaaaggccgattcaccatctccaaaacctcgaccacggtggatctgaaaatcaccagtccgacaaccgaggacacggccacgtatttctgtgccagagggggtgccgatattcatggttatgcttatggtacgttgggtaccttgtggggcccaggcaccctggtcaccgtctcctcaggccagcccaaggcccccagcgtgttccctctggccccctgttgtggcgacaccccctcctccaccgtgaccctgggctgtctggtgaagggctacctgcccgagcccgtgaccgtgacatggaacagcggaaccctgaccaacggcgtgagaaccttcccctccgtgcgccagtcctccggcctgtacagcctgtctagcgtggtgtctgtgaccagcagctctcagccagtgacctgtaacgtggcccaccccgccaccaacaccaaagtggacaaaaccgtggccccctccacctgctccaagcccacctgccccccccctgagctgctgggaggaccttccgtgttcatcttcccccccaaacccaaagacaccctgatgatcagcagaacccccgaggtgacctgcgtggtggtggacgtgagccaggacgaccccgaggtgcagtttacatggtacattaacaacgagcaggtgagaaccgccagaccccccctgcgcgagcagcagttcaacagcaccatcagagtggtgagcaccctgcccatcgcccaccaggattggctgagaggcaaggaattcaagtgcaaagtgcacaacaaggccctgcccgcccccattgagaaaaccatcagcaaagccagaggccagcccctggaacccaaagtgtacaccatggggccccccagagaagaactgagcagcagaagcgtgagcctgacctgcatgatcaacggcttctaccccagcgacatcagcgtggaatgggaaaaaaacggcaaggccgaggacaactacaagaccacccccgccgtgctggacagcgacggcagctacttcctgtacagcaagctgagcgtgcccaccagcgagtggcagagaggcgacgtgttcacctgcagcgtgatgcacgaggccctgcacaaccactacacccagaagagcatcagcagaagccccggcaag

SEQ ID NO: 27 - DNA, 651 bp, synthetic construct
  misc_feature 1..651: note = LC DNA
  source 1..651: mol_type = other DNA
gctgacattgtgatgacccagactccagcctccgtggaggcagctgtgggaggcacagtcaccatcaagtgccaggccagtcagagcattggcactgcattggcctggtatcagcagaaaccagggcagcctcccaagctcctgatctattatgcttccactctggcatctggggtcccatcgcggttcaaaggcagtggatctgggacacagttcactttcaccatcagcgacctggagtgtgccgatgctgccacttactactgtcaatcctattattatagtaacaataatagtgatggttctgctttcggcggagggaccgaggtggtggtcaaaggcgaccccgtggcccccaccgtgctgattttcccccccgccgccgaccaggtggccaccggaaccgtgacaatcgtgtgtgtggccaacaaatacttccccgacgtgaccgtgacatgggaggtggacggaaccacccagaccaccggcatcgaaaacagtaagaccccccagaacagcgccgactgcacctataacctgtccagcacactgaccctgacctctacccagtacaacagccacaaagagtacacctgcaaagtgacacagggcaccaccagcgtggtgcagagcttcaacagaggggactgc

SEQ ID NO: 28 - DNA, 21 bp, synthetic construct
  misc_feature 1..21: note = BI-CMV-F
  source 1..21: mol_type = other DNA
cgcaaatgggcggtaggcgtg

SEQ ID NO: 29 - DNA, 22 bp, synthetic construct
  misc_feature 1..22: note = BI-SEQ-R
  source 1..22: mol_type = other DNA
agcgtaaaaggagcaacatagt